European Patent Application EP 4 538 392 A1, published April 16, 2025. Title: GENETIC SIGNATURE OF LUNG CANCER. Applicant: PANGAEA ONCOLOGY, SA. The sequence listing filed with the application follows.

SEQUENCE LISTING (2 sequences)

SEQ ID NO: 1 - RNA, 100 nt, Homo sapiens
  source 1..100: mol_type = other RNA
gattttgaggacacttgtggagagctcgaattccagaatgatgaaattgttaggttgtgacagttggaagtgtcatgtacaacatgcggcgattaagtct

SEQ ID NO: 2 - RNA, 100 nt, Homo sapiens
  source 1..100: mol_type = other RNA
ctgcttacgagctggtcctggctgatggcagctttgtgcgatgcactccgattgtccgtgtggagcccttggtgaccatgggccaggtgactgccctgct